European Patent Application EP 4 261 285 A1, published October 18, 2023. Title: Neutralizable covalent drug. Applicant: Tabuchi, Yudai Yang, Jay Taki, Masumi. The sequence listing filed with the application follows.

SEQUENCE LISTING (4 sequences)

SEQ ID NO: 1 - DNA, 15 bp, Artificial Sequence
  Thrombin binding aptamer
ggttggtgtggttgg

SEQ ID NO: 2 - DNA, 51 bp, Artificial Sequence
  SARS-CoV-2 spike protein binding aptamer
cagcaccgaccttgtgctttgggagtgctggtccaagggcgttaatggaca

SEQ ID NO: 3 - DNA, 26 bp, Artificial Sequence
  VEGF binding aptamer
caattgggcccgtccgtatggtgggt

SEQ ID NO: 4 - DNA, 15 bp, Artificial Sequence
  Antidote to thrombin binding aptamer
ccaaccacaccaacc